European Patent Specification EP 3 649 158 B1, published May 7, 2025. Title: Split superantigenes and their use for immunotherapy. Applicant: Kemijski institut. The sequence listing filed with the application follows.

SEQUENCE LISTING (6 sequences)

SEQ ID NO: 1 - protein, 120 aa, Staphylococcus aureus
SEKSEEINEKDLRKKSELQGTALGNLKQIYYYNEKAKTENKESHDQFLQHTILFKGFFTDHSWYNDLLVDFDSKDIVDKYKGKKVDLYGAYYGYQCAGGTPNKTACMYGGVTLHDNNRLT

SEQ ID NO: 2 - protein, 122 aa, Staphylococcus aureus
TLHDNNRLTEEKKVPINLWLDGKQNTVPLETVKTNKKNVTVQELDLQARRYLQEKYNLYNSDVFDGKVQRGLIVFHTSTEPSVNYDLFGAQGQYSNTLLRIYRDNKTINSENMHIDIYLYTS

SEQ ID NO: 3 - protein, 33 aa, Artificial sequence
  Artificial sequence
SPEDEIQQLEEEIAQLEQKNAALKEKNQALKYG

SEQ ID NO: 4 - protein, 33 aa, Artificial sequence
  Artificial sequence
SPEDKIAQLKQKIQALKQENQQLEEENAALEYG

SEQ ID NO: 5 - protein, 245 aa, Artificial sequence
  Artificial sequence
QVQLQQSGAEVKKPGSSVKVSCKASGYTFTSYNMHWVKQAPGQGLEWIGAIYPGNGDTSYNQKFKGKATLTADESTNTAYMELSSLRSEDTAFYYCARSTYYGGDWYFDVWGQGTTVTVSSGSTSGSGKPGSGEGSTKGDIQLTQSPSSLSASVGDRVTMTCRASSSVSYIHWFQQKPGKAPKPWIYATSNLASGVPVRFSGSGSGTDYTFTISSLQPEDIATYYCQQWTSNPPTFGGGTKLEIK

SEQ ID NO: 6 - protein, 10 aa, Artificial Sequence
  artifical linker
GGGGSGGGGS